European Patent Specification EP 3 354 729 B1, published February 14, 2024. Title: ANTI-GARP ANTIBODY. Applicant: DAIICHI SANKYO CO. LTD. The sequence listing filed with the application follows.

SEQUENCE LISTING (45 sequences)

SEQ ID NO: 1 - protein, 662 aa, Human
MRPQILLLLALLTLGLAAQHQDKVPCKMVDKKVSCQVLGLLQVPSVLPPDTETLDLSGNQLRSILASPLGFYTALRHLDLSTNEISFLQPGAFQALTHLEHLSLAHNRLAMATALSAGGLGPLPRVTSLDLSGNSLYSGLLERLLGEAPSLHTLSLAENSLTRLTRHTFRDMPALEQLDLHSNVLMDIEDGAFEGLPRLTHLNLSRNSLTCISDFSLQQLRVLDLSCNSIEAFQTASQPQAEFQLTWLDLRENKLLHFPDLAALPRLIYLNLSNNLIRLPTGPPQDSKGIHAPSEGWSALPLSAPSGNASGRPLSQLLNLDLSYNEIELIPDSFLEHLTSLCFLNLSRNCLRTFEARRLGSLPCLMLLDLSHNALETLELGARALGSLRTLLLQGNALRDLPPYTFANLASLQRLNLQGNRVSPCGGPDEPGPSGCVAFSGITSLRSLSLVDNEIELLRAGAFLHTPLTELDLSSNPGLEVATGALGGLEASLEVLALQGNGLMVLQVDLPCFICLKRLNLAENRLSHLPAWTQAVSLEVLDLRNNSFSLLPGSAMGGLETSLRRLYLQGNPLSCCGNGWLAAQLHQGRVDVDATQDLICRFSSQEEVSLSHVRPEDCEKGGLKNINLIIILTFILVSAILLTTLAACCCVRRQKFNQQYKA

SEQ ID NO: 2 - protein, 448 aa, Human
EVQLLESGGGLVQPGGSLRLSCAASGFTFSDYYMSWIRQAPGKGLEWVSGVSWNGSRTHYADSVKGRFTISRDNSKNTLYLQMNSLRAEDTAVYYCARQRQLAEFDYWGQGTLVTVSSASTKGPSVFPLAPSSKSTSGGTAALGCLVKDYFPEPVTVSWNSGALTSGVHTFPAVLQSSGLYSLSSVVTVPSSSLGTQTYICNVNHKPSNTKVDKRVEPKSCDKTHTCPPCPAPELLGGPSVFLFPPKPKDTLMISRTPEVTCVVVDVSHEDPEVKFNWYVDGVEVHNAKTKPREEQYNSTYRVVSVLTVLHQDWLNGKEYKCKVSNKALPAPIEKTISKAKGQPREPQVYTLPPSREEMTKNQVSLTCLVKGFYPSDIAVEWESNGQPENNYKTTPPVLDSDGSFFLYSKLTVDKSRWQQGNVFSCSVMHEALHNHYTQKSLSLSPGK

SEQ ID NO: 3 - protein, 217 aa, Human
QSVLTQPPSASGTPGQRVTISCTGSSSNIGAGYVVHWYQQLPGTAPKLLIYADTNRPSGVPDRFSGSKSGTSASLAISGLRSEDEADYYCQSYDSSLRGWVFGGGTKLTVLGQPKAAPSVTLFPPSSEELQANKATLVCLISDFYPGAVTVAWKADSSPVKAGVETTTPSKQSNNKYAASSYLSLTPEQWKSHRSYSCQVTHEGSTVEKTVAPTECS

SEQ ID NO: 4 - protein, 453 aa, Human
EVQLLESGGGLVQPGGSLRLSCAASGFTFSSYGMHWVRQAPGKGLEWVAGISWNSAITVYADSVKGRFTISRDNSKNTLYLQMNSLRAEDTAVYYCAKDAGGRYSGSYYFDYWGQGTLVTVSSASTKGPSVFPLAPSSKSTSGGTAALGCLVKDYFPEPVTVSWNSGALTSGVHTFPAVLQSSGLYSLSSVVTVPSSSLGTQTYICNVNHKPSNTKVDKRVEPKSCDKTHTCPPCPAPELLGGPSVFLFPPKPKDTLMISRTPEVTCVVVDVSHEDPEVKFNWYVDGVEVHNAKTKPREEQYNSTYRVVSVLTVLHQDWLNGKEYKCKVSNKALPAPIEKTISKAKGQPREPQVYTLPPSREEMTKNQVSLTCLVKGFYPSDIAVEWESNGQPENNYKTTPPVLDSDGSFFLYSKLTVDKSRWQQGNVFSCSVMHEALHNHYTQKSLSLSPGK

SEQ ID NO: 5 - protein, 216 aa, Human
QSVLTQPPSASGTPGQRVTISCTGSSSNIGAGYDVHWYQQLPGTAPKLLIYGNSNRPSGVPDRFSGSKSGTSASLAISGLRSEDEADYYCQSYDRSLNWVFGGGTKLTVLGQPKAAPSVTLFPPSSEELQANKATLVCLISDFYPGAVTVAWKADSSPVKAGVETTTPSKQSNNKYAASSYLSLTPEQWKSHRSYSCQVTHEGSTVEKTVAPTECS

SEQ ID NO: 6 - DNA, 1344 bp, Human
gaggtgcagctgttggagtctgggggaggcttggtacagcctggggggtccctgagactctcctgtgcagcctctggattcaccttcagtgactactacatgagctggatccgccaggctccaggcaaggggctggagtgggtatcgggtgttagttggaatggcagtaggacgcactatgcagactctgtgaagggccgattcaccatctccagagacaattccaagaacacgctgtatctgcaaatgaacagcctgagagccgaggacactgccgtgtattactgtgccagacagaggcagctggctgaatttgactactggggccaaggtaccctggtcaccgtgagctcagcctccaccaagggcccaagcgtcttccccctggcaccctcctccaagagcacctctggcggcacagccgccctgggctgcctggtcaaggactacttccccgaacccgtgaccgtgagctggaactcaggcgccctgaccagcggcgtgcacaccttccccgctgtcctgcagtcctcaggactctactccctcagcagcgtggtgaccgtgccctccagcagcttgggcacccagacctacatctgcaacgtgaatcacaagcccagcaacaccaaggtggacaagagagttgagcccaaatcttgtgacaaaactcacacatgcccaccctgcccagcacctgaactcctggggggaccctcagtcttcctcttccccccaaaacccaaggacaccctcatgatctcccggacccctgaggtcacatgcgtggtggtggacgtgagccacgaagaccctgaggtcaagttcaactggtacgtggacggcgtggaggtgcataatgccaagacaaagccccgggaggagcagtacaacagcacgtaccgggtggtcagcgtcctcaccgtcctgcaccaggactggctgaatggcaaggagtacaagtgcaaggtctccaacaaagccctcccagcccccatcgagaaaaccatctccaaagccaaaggccagccccgggaaccacaggtgtacaccctgcccccatcccgggaggagatgaccaagaaccaggtcagcctgacctgcctggtcaaaggcttctatcccagcgacatcgccgtggagtgggagagcaatggccagcccgagaacaactacaagaccacccctcccgtgctggactccgacggctccttcttcctctacagcaagctcaccgtggacaagagcaggtggcagcagggcaacgtcttctcatgctccgtgatgcatgaggctctgcacaaccactacacccagaagagcctctccctgtctcccggcaaa

SEQ ID NO: 7 - DNA, 651 bp, Human
cagtctgtgctgactcagccaccctcagcgtctgggacccccgggcagagggtcaccatctcctgcactgggagcagctccaacattggggcgggttatgttgtacattggtatcagcagctcccaggaacggcccccaaactcctcatctatgctgacaccaatcggccctcaggggtccctgaccgattctctggctccaagtctggcacctcagcctccctggccatcagtgggctccggtccgaggatgaggctgattattactgccagtcctatgacagcagcctgagaggttgggtgttcggcggaggaaccaagctgacggtcctaggtcagcctaaggctgcccctagcgtgaccctgttccctccttccagcgaggagcttcaagctaacaaggccaccctggtgtgtcttatctctgacttctaccctggcgctgtgaccgtggcctggaaggctgacagctcccctgtgaaggccggagtggagaccaccacacctagcaagcagtctaacaacaagtacgctgccagctcctacctgagccttacccctgagcagtggaagtctcacagaagctactcctgtcaagtgacccacgagggcagcaccgtggagaagaccgtggctcctaccgagtgttcc

SEQ ID NO: 8 - DNA, 1359 bp, Human
gaggtgcagctgttggagtctgggggaggcttggtacagcctggggggtccctgagactctcctgtgcagcctctggattcaccttcagtagctatggcatgcactgggtccgccaggctccaggcaaggggctggagtgggtcgccggaattagttggaacagtgccatcacagtctatgcggactctgtgaagggccggttcaccatctccagagacaattccaagaacacgctgtatctgcaaatgaacagcctgagagccgaggacactgccgtgtattactgtgcaaaagatgccgggggccggtatagtgggagctactactttgactactggggccaaggtaccctggtcaccgtgagctcagcctccaccaagggcccaagcgtcttccccctggcaccctcctccaagagcacctctggcggcacagccgccctgggctgcctggtcaaggactacttccccgaacccgtgaccgtgagctggaactcaggcgccctgaccagcggcgtgcacaccttccccgctgtcctgcagtcctcaggactctactccctcagcagcgtggtgaccgtgccctccagcagcttgggcacccagacctacatctgcaacgtgaatcacaagcccagcaacaccaaggtggacaagagagttgagcccaaatcttgtgacaaaactcacacatgcccaccctgcccagcacctgaactcctggggggaccctcagtcttcctcttccccccaaaacccaaggacaccctcatgatctcccggacccctgaggtcacatgcgtggtggtggacgtgagccacgaagaccctgaggtcaagttcaactggtacgtggacggcgtggaggtgcataatgccaagacaaagccccgggaggagcagtacaacagcacgtaccgggtggtcagcgtcctcaccgtcctgcaccaggactggctgaatggcaaggagtacaagtgcaaggtctccaacaaagccctcccagcccccatcgagaaaaccatctccaaagccaaaggccagccccgggaaccacaggtgtacaccctgcccccatcccgggaggagatgaccaagaaccaggtcagcctgacctgcctggtcaaaggcttctatcccagcgacatcgccgtggagtgggagagcaatggccagcccgagaacaactacaagaccacccctcccgtgctggactccgacggctccttcttcctctacagcaagctcaccgtggacaagagcaggtggcagcagggcaacgtcttctcatgctccgtgatgcatgaggctctgcacaaccactacacccagaagagcctctccctgtctcccggcaaa

SEQ ID NO: 9 - DNA, 648 bp, Human
cagtctgtgctgactcagccaccctcagcgtctgggacccccgggcagagggtcaccatctcctgcactgggagcagctccaacatcggggcaggttatgatgtacactggtatcagcagctcccaggaacggcccccaaactcctcatctatggtaacagcaatcggccctcaggggtccctgaccgattctctggctccaagtctggcacctcagcctccctggccatcagtgggctccggtccgaggatgaggctgattattactgccagtcctatgacagaagcctgaattgggtgttcggcggaggaaccaagctgacggtcctaggtcagcctaaggctgcccctagcgtgaccctgttccctccttccagcgaggagcttcaagctaacaaggccaccctggtgtgtcttatctctgacttctaccctggcgctgtgaccgtggcctggaaggctgacagctcccctgtgaaggccggagtggagaccaccacacctagcaagcagtctaacaacaagtacgctgccagctcctacctgagccttacccctgagcagtggaagtctcacagaagctactcctgtcaagtgacccacgagggcagcaccgtggagaagaccgtggctcctaccgagtgttcc

SEQ ID NO: 10 - DNA, 24 bp, Artificial Sequence
  Primer A
gaaacagctatgaaatacctattg

SEQ ID NO: 11 - DNA, 19 bp, Artificial Sequence
  Primer B
gcctgagcagtggaagtcc

SEQ ID NO: 12 - DNA, 24 bp, Artificial Sequence
  Primer C
taggtatttcattatgactgtctc

SEQ ID NO: 13 - DNA, 23 bp, Artificial Sequence
  Primer D
cccagtcacgacgttgtaaaacg

SEQ ID NO: 14 - DNA, 351 bp, Rat
gaggtgcagctggtggagtctgggggaggcttagtgcagcctggaaggtccaagaaactctcctgttcagcctcaggattcactttcagtaactattacatggcctgggtccgccaggctccaacgcagggtctggagtgggtcgcatccattggtactgttggtggtaacacttactatcgagactccgtgaagggccgattcactatctccagagatgatgcaaaaagcaccctatacctgcaaatggacagtctgaggtctgaggacacggccacttattactgtgcaagagaggattacggagggtttccccactggggccaaggagtcatggtcacagtctcctca

SEQ ID NO: 15 - protein, 117 aa, Rat
EVQLVESGGGLVQPGRSKKLSCSASGFTFSNYYMAWVRQAPTQGLEWVASIGTVGGNTYYRDSVKGRFTISRDDAKSTLYLQMDSLRSEDTATYYCAREDYGGFPHWGQGVMVTVSS

SEQ ID NO: 16 - DNA, 327 bp, Rat
aatattgtgatgactcagtctcccacatccatgttcatatcagtcggagacagggtcaccatgaactgtaaggccagtcagaatgtgggaactaatgtagactggtaccagcagaaaacagggcagtctcctaaactgcttatctatggggcgtccaaccgctacactggagtccctgatcgcttcacaggcagtggatctggaacagatttcactctcaccatcagcaacatgcaggctgaagacctggctgtttatgactgtctacagtataagtacaatccatacacgtttggaactgggaccaagctggaactgaaccgggct

SEQ ID NO: 17 - protein, 109 aa, Rat
NIVMTQSPTSMFISVGDRVTMNCKASQNVGTNVDWYQQKTGQSPKLLIYGASNRYTGVPDRFTGSGSGTDFTLTISNMQAEDLAVYDCLQYKYNPYTFGTGTKLELNRA

SEQ ID NO: 18 - DNA, 360 bp, Rat
caggtgcagctgagggagtcaggacctggtctggtgcagccctcacagaccctgtccctcacctgcactgtctctgggttctcactaaccagctttcatgtaagctgggttcgccagcctccagagaagggtctggagtggattgcaacaatttcaagtggtggaggtacatattataattcagctctcaaatcccgactgagcatcagcagggacacctccaagagccaagttttcttaaagatgagcactctgcaaactgaagacacagccatgtacttctgtgcccggatttcgggctggggccattactatgttatggatgtctggggtcaaggagcttcagtcactgtctcctca

SEQ ID NO: 19 - protein, 120 aa, Rat
QVQLRESGPGLVQPSQTLSLTCTVSGFSLTSFHVSWVRQPPEKGLEWIATISSGGGTYYNSALKSRLSISRDTSKSQVFLKMSTLQTEDTAMYFCARISGWGHYYVMDVWGQGASVTVSS

SEQ ID NO: 20 - DNA, 327 bp, Rat
gacatccagatgacacagtctccagcttccctgtctggatctctgggagaaactgtcaccatccaatgtcaagcaagtgaggacatttacagtggtttagcgtggtatcagcagaagccagggaaatctcctcagctcctgatctatggtgcaggtagcttacaagacggcgtcccatcacgattcagtggcggtggatctggcacacattattctctcaagatcagcagcatgcaaactgaagatgaaggggtttatttctgtcaacagggtttaaagtttccgctcacgttcggttctgggaccaagctggagatcaaacgggct

SEQ ID NO: 21 - protein, 109 aa, Rat
DIQMTQSPASLSGSLGETVTIQCQASEDIYSGLAWYQQKPGKSPQLLIYGAGSLQDGVPSRFSGGGSGTHYSLKISSMQTEDEGVYFCQQGLKFPLTFGSGTKLEIKRA

SEQ ID NO: 22 - DNA, 449 bp, Human
gcctccggactctagagccaccatggtgctgcagacccaggtgttcatctccctgctgctgtggatctccggcgcgtacggcgatatcgtgatgattaaacgtacggtggccgccccctccgtgttcatcttccccccctccgacgagcagctgaagtccggcaccgcctccgtggtgtgcctgctgaataacttctaccccagagaggccaaggtgcagtggaaggtggacaacgccctgcagtccgggaactcccaggagagcgtgaccgagcaggacagcaaggacagcacctacagcctgagcagcaccctgaccctgagcaaagccgactacgagaagcacaaggtgtacgcctgcgaggtgacccaccagggcctgagctcccccgtcaccaagagcttcaacaggggggagtgttaggggcccgtttaaacgggggaggcta

SEQ ID NO: 23 - DNA, 1132 bp, Human
gcctccggactctagagccaccatgaaacacctgtggttcttcctcctgctggtggcagctcccagatgggtgctgagccaggtgcaattgtgcaggcggttagctcagcctccaccaagggcccaagcgtcttccccctggcaccctcctccaagagcacctctggcggcacagccgccctgggctgcctggtcaaggactacttccccgaacccgtgaccgtgagctggaactcaggcgccctgaccagcggcgtgcacaccttccccgctgtcctgcagtcctcaggactctactccctcagcagcgtggtgaccgtgccctccagcagcttgggcacccagacctacatctgcaacgtgaatcacaagcccagcaacaccaaggtggacaagagagttgagcccaaatcttgtgacaaaactcacacatgcccaccctgcccagcacctgaactcctggggggaccctcagtcttcctcttccccccaaaacccaaggacaccctcatgatctcccggacccctgaggtcacatgcgtggtggtggacgtgagccacgaagaccctgaggtcaagttcaactggtacgtggacggcgtggaggtgcataatgccaagacaaagccccgggaggagcagtacaacagcacgtaccgggtggtcagcgtcctcaccgtcctgcaccaggactggctgaatggcaaggagtacaagtgcaaggtctccaacaaagccctcccagcccccatcgagaaaaccatctccaaagccaaaggccagccccgggaaccacaggtgtacaccctgcccccatcccgggaggagatgaccaagaaccaggtcagcctgacctgcctggtcaaaggcttctatcccagcgacatcgccgtggagtgggagagcaatggccagcccgagaacaactacaagaccacccctcccgtgctggactccgacggctccttcttcctctacagcaagctcaccgtggacaagagcaggtggcagcagggcaacgtcttctcatgctccgtgatgcatgaggctctgcacaaccactacacccagaagagcctctccctgtctcccggcaaatgagatatcgggcccgtttaaacgggggaggcta

SEQ ID NO: 24 - DNA, 1398 bp, Artificial Sequence
  Chimeric Antibody
atgaaacacctgtggttcttcctcctgctggtggcagctcccagatgggtgctgagcgaggtgcagctggtggagtctgggggaggcttagtgcagcctggaaggtccaagaaactctcctgttcagcctcaggattcactttcagtaactattacatggcctgggtccgccaggctccaacgcagggtctggagtgggtcgcatccattggtactgttggtggtaacacttactatcgagactccgtgaagggccgattcactatctccagagatgatgcaaaaagcaccctatacctgcaaatggacagtctgaggtctgaggacacggccacttattactgtgcaagagaggattacggagggtttccccactggggccaaggagtcatggtcacagtcagctcagcctccaccaagggcccaagcgtcttccccctggcaccctcctccaagagcacctctggcggcacagccgccctgggctgcctggtcaaggactacttccccgaacccgtgaccgtgagctggaactcaggcgccctgaccagcggcgtgcacaccttccccgctgtcctgcagtcctcaggactctactccctcagcagcgtggtgaccgtgccctccagcagcttgggcacccagacctacatctgcaacgtgaatcacaagcccagcaacaccaaggtggacaagagagttgagcccaaatcttgtgacaaaactcacacatgcccaccctgcccagcacctgaactcctggggggaccctcagtcttcctcttccccccaaaacccaaggacaccctcatgatctcccggacccctgaggtcacatgcgtggtggtggacgtgagccacgaagaccctgaggtcaagttcaactggtacgtggacggcgtggaggtgcataatgccaagacaaagccccgggaggagcagtacaacagcacgtaccgggtggtcagcgtcctcaccgtcctgcaccaggactggctgaatggcaaggagtacaagtgcaaggtctccaacaaagccctcccagcccccatcgagaaaaccatctccaaagccaaaggccagccccgggaaccacaggtgtacaccctgcccccatcccgggaggagatgaccaagaaccaggtcagcctgacctgcctggtcaaaggcttctatcccagcgacatcgccgtggagtgggagagcaatggccagcccgagaacaactacaagaccacccctcccgtgctggactccgacggctccttcttcctctacagcaagctcaccgtggacaagagcaggtggcagcagggcaacgtcttctcatgctccgtgatgcatgaggctctgcacaaccactacacccagaagagcctctccctgtctcccggcaaa

SEQ ID NO: 25 - protein, 466 aa, Artificial Sequence
  Chimeric Antibody
MKHLWFFLLLVAAPRWVLSEVQLVESGGGLVQPGRSKKLSCSASGFTFSNYYMAWVRQAPTQGLEWVASIGTVGGNTYYRDSVKGRFTISRDDAKSTLYLQMDSLRSEDTATYYCAREDYGGFPHWGQGVMVTVSSASTKGPSVFPLAPSSKSTSGGTAALGCLVKDYFPEPVTVSWNSGALTSGVHTFPAVLQSSGLYSLSSVVTVPSSSLGTQTYICNVNHKPSNTKVDKRVEPKSCDKTHTCPPCPAPELLGGPSVFLFPPKPKDTLMISRTPEVTCVVVDVSHEDPEVKFNWYVDGVEVHNAKTKPREEQYNSTYRVVSVLTVLHQDWLNGKEYKCKVSNKALPAPIEKTISKAKGQPREPQVYTLPPSREEMTKNQVSLTCLVKGFYPSDIAVEWESNGQPENNYKTTPPVLDSDGSFFLYSKLTVDKSRWQQGNVFSCSVMHEALHNHYTQKSLSLSPGK

SEQ ID NO: 26 - DNA, 702 bp, Artificial Sequence
  Chimeric Antibody
atggtgctgcagacccaggtgttcatctccctgctgctgtggatctccggcgcgtacggcaatattgtgatgactcagtctcccacatccatgttcatatcagtcggagacagggtcaccatgaactgtaaggccagtcagaatgtgggaactaatgtagactggtaccagcagaaaacagggcagtctcctaaactgcttatctatggggcgtccaaccgctacactggagtccctgatcgcttcacaggcagtggatctggaacagatttcactctcaccatcagcaacatgcaggctgaagacctggctgtttatgactgtctacagtataagtacaatccatacacgtttggaactgggaccaagctggaactgaaccgggctgtggccgccccctccgtgttcatcttccccccctccgacgagcagctgaagtccggcaccgcctccgtggtgtgcctgctgaataacttctaccccagagaggccaaggtgcagtggaaggtggacaacgccctgcagtccgggaactcccaggagagcgtgaccgagcaggacagcaaggacagcacctacagcctgagcagcaccctgaccctgagcaaagccgactacgagaagcacaaggtgtacgcctgcgaggtgacccaccagggcctgagctcccccgtcaccaagagcttcaacaggggggagtgt

SEQ ID NO: 27 - protein, 234 aa, Artificial Sequence
  Chimeric Antibody
MVLQTQVFISLLLWISGAYGNIVMTQSPTSMFISVGDRVTMNCKASQNVGTNVDWYQQKTGQSPKLLIYGASNRYTGVPDRFTGSGSGTDFTLTISNMQAEDLAVYDCLQYKYNPYTFGTGTKLELNRAVAAPSVFIFPPSDEQLKSGTASVVCLLNNFYPREAKVQWKVDNALQSGNSQESVTEQDSKDSTYSLSSTLTLSKADYEKHKVYACEVTHQGLSSPVTKSFNRGEC

SEQ ID NO: 28 - DNA, 1407 bp, Artificial Sequence
  Chimeric Antibody
atgaaacacctgtggttcttcctcctgctggtggcagctcccagatgggtgctgagccaggtgcagctgagggagtcaggacctggtctggtgcagccctcacagaccctgtccctcacctgcactgtctctgggttctcactaaccagctttcatgtaagctgggttcgccagcctccagagaagggtctggagtggattgcaacaatttcaagtggtggaggtacatattataattcagctctcaaatcccgactgagcatcagcagggacacctccaagagccaagttttcttaaagatgagcactctgcaaactgaagacacagccatgtacttctgtgcccggatttcgggctggggccattactatgttatggatgtctggggtcaaggagcttcagtcactgtcagctcagcctccaccaagggcccaagcgtcttccccctggcaccctcctccaagagcacctctggcggcacagccgccctgggctgcctggtcaaggactacttccccgaacccgtgaccgtgagctggaactcaggcgccctgaccagcggcgtgcacaccttccccgctgtcctgcagtcctcaggactctactccctcagcagcgtggtgaccgtgccctccagcagcttgggcacccagacctacatctgcaacgtgaatcacaagcccagcaacaccaaggtggacaagagagttgagcccaaatcttgtgacaaaactcacacatgcccaccctgcccagcacctgaactcctggggggaccctcagtcttcctcttccccccaaaacccaaggacaccctcatgatctcccggacccctgaggtcacatgcgtggtggtggacgtgagccacgaagaccctgaggtcaagttcaactggtacgtggacggcgtggaggtgcataatgccaagacaaagccccgggaggagcagtacaacagcacgtaccgggtggtcagcgtcctcaccgtcctgcaccaggactggctgaatggcaaggagtacaagtgcaaggtctccaacaaagccctcccagcccccatcgagaaaaccatctccaaagccaaaggccagccccgggaaccacaggtgtacaccctgcccccatcccgggaggagatgaccaagaaccaggtcagcctgacctgcctggtcaaaggcttctatcccagcgacatcgccgtggagtgggagagcaatggccagcccgagaacaactacaagaccacccctcccgtgctggactccgacggctccttcttcctctacagcaagctcaccgtggacaagagcaggtggcagcagggcaacgtcttctcatgctccgtgatgcatgaggctctgcacaaccactacacccagaagagcctctccctgtctcccggcaaa

SEQ ID NO: 29 - protein, 469 aa, Artificial Sequence
  Chimeric Antibody
MKHLWFFLLLVAAPRWVLSQVQLRESGPGLVQPSQTLSLTCTVSGFSLTSFHVSWVRQPPEKGLEWIATISSGGGTYYNSALKSRLSISRDTSKSQVFLKMSTLQTEDTAMYFCARISGWGHYYVMDVWGQGASVTVSSASTKGPSVFPLAPSSKSTSGGTAALGCLVKDYFPEPVTVSWNSGALTSGVHTFPAVLQSSGLYSLSSVVTVPSSSLGTQTYICNVNHKPSNTKVDKRVEPKSCDKTHTCPPCPAPELLGGPSVFLFPPKPKDTLMISRTPEVTCVVVDVSHEDPEVKFNWYVDGVEVHNAKTKPREEQYNSTYRVVSVLTVLHQDWLNGKEYKCKVSNKALPAPIEKTISKAKGQPREPQVYTLPPSREEMTKNQVSLTCLVKGFYPSDIAVEWESNGQPENNYKTTPPVLDSDGSFFLYSKLTVDKSRWQQGNVFSCSVMHEALHNHYTQKSLSLSPGK

SEQ ID NO: 30 - DNA, 702 bp, Artificial Sequence
  Chimeric Antibody
atggtgctgcagacccaggtgttcatctccctgctgctgtggatctccggcgcgtacggcgacatccagatgacacagtctccagcttccctgtctggatctctgggagaaactgtcaccatccaatgtcaagcaagtgaggacatttacagtggtttagcgtggtatcagcagaagccagggaaatctcctcagctcctgatctatggtgcaggtagcttacaagacggcgtcccatcacgattcagtggcggtggatctggcacacattattctctcaagatcagcagcatgcaaactgaagatgaaggggtttatttctgtcaacagggtttaaagtttccgctcacgttcggttctgggaccaagctggagatcaaacgggctgtggccgccccctccgtgttcatcttccccccctccgacgagcagctgaagtccggcaccgcctccgtggtgtgcctgctgaataacttctaccccagagaggccaaggtgcagtggaaggtggacaacgccctgcagtccgggaactcccaggagagcgtgaccgagcaggacagcaaggacagcacctacagcctgagcagcaccctgaccctgagcaaagccgactacgagaagcacaaggtgtacgcctgcgaggtgacccaccagggcctgagctcccccgtcaccaagagcttcaacaggggggagtgt

SEQ ID NO: 31 - protein, 234 aa, Artificial Sequence
  Chimeric Antibody
MVLQTQVFISLLLWISGAYGDIQMTQSPASLSGSLGETVTIQCQASEDIYSGLAWYQQKPGKSPQLLIYGAGSLQDGVPSRFSGGGSGTHYSLKISSMQTEDEGVYFCQQGLKFPLTFGSGTKLEIKRAVAAPSVFIFPPSDEQLKSGTASVVCLLNNFYPREAKVQWKVDNALQSGNSQESVTEQDSKDSTYSLSSTLTLSKADYEKHKVYACEVTHQGLSSPVTKSFNRGEC

SEQ ID NO: 32 - DNA, 1398 bp, Artificial Sequence
  Humanized Antibody
atgaagcacctgtggttctttctgctgctggtggccgctcccagatgggtgctgtctgaagtgcagctggtggaatccggcggaggcctggtgcagcctggcggatctctgagactgtcttgtgccgcctccggcttcaccttctccaactactacatggcctgggtgcgacaggcccctggcaagggactggaatgggtgtcctctatcggcaccgtgggcggcaacacctactacgccgattctgtgaagggccggttcaccatctcccgggacgactccaagaacaccctgtacctgcagatgaactccctgcgggccgaggacaccgccgtgtactactgtgccagagaggactacggcggcttccctcattggggccagggcacactcgtgaccgtgtcctctgcttccaccaagggcccctccgtgtttcctctggccccttccagcaagtccacctctggcggaacagccgctctgggctgcctcgtgaaggactacttccccgagcccgtgacagtgtcttggaactctggcgccctgacctccggcgtgcacacctttccagctgtgctgcagtcctccggcctgtactccctgtcctccgtcgtgactgtgccctccagctctctgggcacccagacctacatctgcaacgtgaaccacaagccctccaacaccaaggtggacaagcgggtggaacccaagtcctgcgacaagacccacacctgtcccccttgtcctgcccctgaactgctgggcggaccttccgtgttcctgttccccccaaagcctaaggacaccctgatgatctcccggacccccgaagtgacctgcgtggtggtggatgtgtcccacgaggaccctgaagtgaagttcaattggtacgtggacggcgtggaagtgcacaacgccaagaccaagcctagagaggaacagtacaactccacctaccgggtggtgtccgtgctgaccgtgctgcatcaggactggctgaacggcaaagagtacaagtgcaaggtgtccaacaaggccctgcctgcccccatcgaaaagaccatctccaaggccaagggccagccccgggaaccccaggtgtacacactgccccctagccgggaagagatgaccaagaaccaggtgtccctgacctgtctcgtgaaaggcttctacccctccgatatcgccgtggaatgggagagcaacggccagcccgagaacaactacaagaccaccccccctgtgctggactccgacggctcattcttcctgtacagcaagctgacagtggacaagtcccggtggcagcagggcaacgtgttctcctgctccgtgatgcacgaggccctgcacaaccactacacccagaagtccctgtccctgagccccggcaaa

SEQ ID NO: 33 - protein, 466 aa, Artificial Sequence
  Humanized Antibody
MKHLWFFLLLVAAPRWVLSEVQLVESGGGLVQPGGSLRLSCAASGFTFSNYYMAWVRQAPGKGLEWVSSIGTVGGNTYYADSVKGRFTISRDDSKNTLYLQMNSLRAEDTAVYYCAREDYGGFPHWGQGTLVTVSSASTKGPSVFPLAPSSKSTSGGTAALGCLVKDYFPEPVTVSWNSGALTSGVHTFPAVLQSSGLYSLSSVVTVPSSSLGTQTYICNVNHKPSNTKVDKRVEPKSCDKTHTCPPCPAPELLGGPSVFLFPPKPKDTLMISRTPEVTCVVVDVSHEDPEVKFNWYVDGVEVHNAKTKPREEQYNSTYRVVSVLTVLHQDWLNGKEYKCKVSNKALPAPIEKTISKAKGQPREPQVYTLPPSREEMTKNQVSLTCLVKGFYPSDIAVEWESNGQPENNYKTTPPVLDSDGSFFLYSKLTVDKSRWQQGNVFSCSVMHEALHNHYTQKSLSLSPGK

SEQ ID NO: 34 - DNA, 1398 bp, Artificial Sequence
  Humanized Antibody
atgaagcacctgtggttctttctgctgctggtggccgctcccagatgggtgctgtctgaagtgcagctggtggaatccggcggaggcctggtgcagcctggcggatctctgagactgtcttgtgccgcctccggcttcaccttctccaactactacatggcctgggtgcgacaggcccctggcaagggactggaatgggtggcctctatcggcaccgtgggcggcaacacctactaccgggattctgtgaagggccggttcaccatctcccgggacgactccaagtccaccctgtacctgcagatgaactccctgcgggccgaggacaccgccgtgtactactgtgccagagaggactacggcggcttccctcattggggccagggcacactcgtgaccgtgtcctctgcttccaccaagggcccctccgtgtttcctctggccccttccagcaagtctacctccggcggaacagccgctctgggctgcctcgtgaaggactacttccccgagcccgtgacagtgtcttggaactctggcgccctgaccagcggcgtgcacacctttccagctgtgctgcagtcctccggcctgtactccctgtcctccgtcgtgactgtgccctccagctctctgggcacccagacctacatctgcaacgtgaaccacaagccctccaacaccaaggtggacaagcgggtggaacccaagtcctgcgacaagacccacacctgtcccccttgtcctgcccctgaactgctgggcggaccttccgtgttcctgttccccccaaagcccaaggacaccctgatgatctcccggacccccgaagtgacctgcgtggtggtggatgtgtcccacgaggaccctgaagtgaagttcaattggtacgtggacggcgtggaagtgcacaacgccaagaccaagcctagagaggaacagtacaactccacctaccgggtggtgtccgtgctgaccgtgctgcatcaggactggctgaacggcaaagagtacaagtgcaaggtgtccaacaaggccctgcctgcccccatcgaaaagaccatctccaaggccaagggccagccccgggaaccccaggtgtacacactgccccctagccgggaagagatgaccaagaaccaggtgtccctgacctgtctcgtgaaaggcttctacccctccgatatcgccgtggaatgggagtccaacggccagcctgagaacaactacaagaccaccccccctgtgctggactccgacggctcattcttcctgtacagcaagctgacagtggacaagtcccggtggcagcagggcaacgtgttctcctgctccgtgatgcacgaggccctgcacaaccactacacccagaagtccctgtccctgagccccggcaaa

SEQ ID NO: 35 - protein, 466 aa, Artificial Sequence
  Humanized Antibody
MKHLWFFLLLVAAPRWVLSEVQLVESGGGLVQPGGSLRLSCAASGFTFSNYYMAWVRQAPGKGLEWVASIGTVGGNTYYRDSVKGRFTISRDDSKSTLYLQMNSLRAEDTAVYYCAREDYGGFPHWGQGTLVTVSSASTKGPSVFPLAPSSKSTSGGTAALGCLVKDYFPEPVTVSWNSGALTSGVHTFPAVLQSSGLYSLSSVVTVPSSSLGTQTYICNVNHKPSNTKVDKRVEPKSCDKTHTCPPCPAPELLGGPSVFLFPPKPKDTLMISRTPEVTCVVVDVSHEDPEVKFNWYVDGVEVHNAKTKPREEQYNSTYRVVSVLTVLHQDWLNGKEYKCKVSNKALPAPIEKTISKAKGQPREPQVYTLPPSREEMTKNQVSLTCLVKGFYPSDIAVEWESNGQPENNYKTTPPVLDSDGSFFLYSKLTVDKSRWQQGNVFSCSVMHEALHNHYTQKSLSLSPGK

SEQ ID NO: 36 - DNA, 702 bp, Artificial Sequence
  Humanized Antibody
atggtgctgcagacccaggtgttcatctccctgctgctgtggatctccggcgcctacggcaacatcgtgatgacccagtcccccgactccctggctgtgtctctgggcgagagagccaccatcaactgcaaggcctcccagaacgtgggcaccaacgtggactggtatcagcagaagcccggccagtcccctaagctgctgatctacggcgccagcaaccggtacaccggcgtgcccgatagattctccggctctggctctggcaccgactttaccctgacaatcagctctctgcaggccgaggacgtggccgtgtacgactgcctgcagtacaagtacaacccctacaccttcggccagggcacaaaggtggaaatcaagcggaccgtggccgctccctccgtgtttatcttcccaccctccgacgagcagctgaagtccggcacagcttccgtcgtgtgcctgctgaacaacttctacccccgcgaggccaaggtgcagtggaaggtggacaacgccctgcagtccggcaactcccaggaatccgtgaccgagcaggactccaaggacagcacctactccctgtcctccaccctgaccctgtccaaggccgactacgagaagcacaaggtgtacgcctgcgaagtgacccaccagggcctgtctagccccgtgaccaagtctttcaaccggggcgagtgc

SEQ ID NO: 37 - protein, 234 aa, Artificial Sequence
  Humanized Antibody
MVLQTQVFISLLLWISGAYGNIVMTQSPDSLAVSLGERATINCKASQNVGTNVDWYQQKPGQSPKLLIYGASNRYTGVPDRFSGSGSGTDFTLTISSLQAEDVAVYDCLQYKYNPYTFGQGTKVEIKRTVAAPSVFIFPPSDEQLKSGTASVVCLLNNFYPREAKVQWKVDNALQSGNSQESVTEQDSKDSTYSLSSTLTLSKADYEKHKVYACEVTHQGLSSPVTKSFNRGEC

SEQ ID NO: 38 - DNA, 702 bp, Artificial Sequence
  Humanized Antibod
atggtgctgcagacccaggtgttcatctccctgctgctgtggatctccggcgcctacggcaacatcgtgatgacccagtccccctccagcctgtctgcttccgtgggcgacagagtgaccatcaactgcaaggcctcccagaacgtgggcaccaacgtggactggtatcagcagaagcccggcaagtcccccaagctgctgatctacggcgccagcaacagatacaccggcgtgcccgacagattctccggctctggctctggcaccgactttaccctgaccatcagctccctgcagcccgaggacttcgccacctacgactgcctgcagtacaagtacaacccctacaccttcggccagggcacaaaggtggaaatcaagcggaccgtggccgctccctccgtgtttatcttcccaccctccgacgagcagctgaagtccggcacagcttctgtcgtgtgcctgctgaacaacttctacccccgcgaggccaaggtgcagtggaaggtggacaacgccctgcagtccggcaactcccaggaatccgtgaccgagcaggactccaaggacagcacctactccctgtcctccaccctgaccctgtccaaggccgactacgagaagcacaaggtgtacgcctgcgaagtgacccaccagggcctgtctagccccgtgaccaagtctttcaaccggggcgagtgc

SEQ ID NO: 39 - protein, 234 aa, Artificial Sequence
  Humanized Antibody
MVLQTQVFISLLLWISGAYGNIVMTQSPSSLSASVGDRVTINCKASQNVGTNVDWYQQKPGKSPKLLIYGASNRYTGVPDRFSGSGSGTDFTLTISSLQPEDFATYDCLQYKYNPYTFGQGTKVEIKRTVAAPSVFIFPPSDEQLKSGTASVVCLLNNFYPREAKVQWKVDNALQSGNSQESVTEQDSKDSTYSLSSTLTLSKADYEKHKVYACEVTHQGLSSPVTKSFNRGEC

SEQ ID NO: 40 - DNA, 1407 bp, Artificial Sequence
  Humanized Antibody
atgaagcacctgtggttctttctgctgctggtggccgctcccagatgggtgctgtctgaagtgcagctggtggaatccggcggaggcctcgtgaagccttcccagaccctgtctctgacctgcaccgtgtccggcttctccctgacctccttccacgtgtcatgggtgcgacagcctccaggcaagggcctggaatggatcgccaccatctcctctggcggcggaacctactacaaccccagcctgaagtccagagtgaccatctcccgggacacctccaagaaccaggtgtccctgaagctgtcctccgtgaccgccgctgataccgccgtgtactactgcgccagaatctccggctggggccactactacgtgatggacgtgtggggccagggcaccctcgtgacagtgtcctctgcttccaccaagggcccctccgtgtttcctctggccccttccagcaagtctacctccggcggaacagccgctctgggctgcctcgtgaaagactacttccccgagcccgtgaccgtgtcttggaactctggcgctctgaccagcggcgtgcacacctttccagctgtgctgcagtcctccggcctgtactccctgtccagcgtcgtgactgtgccctccagctctctgggcacccagacctacatctgcaacgtgaaccacaagccctccaacaccaaggtggacaagcgggtggaacccaagtcctgcgacaagacccacacctgtcccccttgtcctgcccctgaactgctgggcggaccttccgtgttcctgttccccccaaagcccaaggacaccctgatgatctcccggacccccgaagtgacctgcgtggtggtggatgtgtcccacgaggaccctgaagtgaagttcaattggtacgtggacggcgtggaagtgcacaacgccaagaccaagcctagagaggaacagtacaactccacctaccgggtggtgtccgtgctgaccgtgctgcaccaggattggctgaacggcaaagagtacaagtgcaaggtgtccaacaaggccctgcctgcccccatcgaaaagaccatcagcaaggccaagggccagccccgggaaccccaggtgtacacactgccccctagccgggaagagatgacaaaaaatcaggtgtcactgacctgtctcgtgaagggcttctacccctccgatatcgccgtggaatgggagtccaacggccagcctgagaacaactacaagaccaccccccctgtgctggactccgacggctcattcttcctgtacagcaagctgacagtggacaagtcccggtggcagcagggcaacgtgttctcctgctccgtgatgcacgaggccctgcacaaccactacacccagaagtccctgtccctgagccccggcaaa

SEQ ID NO: 41 - protein, 469 aa, Artificial Sequence
  Humanized Antibody
MKHLWFFLLLVAAPRWVLSEVQLVESGGGLVKPSQTLSLTCTVSGFSLTSFHVSWVRQPPGKGLEWIATISSGGGTYYNPSLKSRVTISRDTSKNQVSLKLSSVTAADTAVYYCARISGWGHYYVMDVWGQGTLVTVSSASTKGPSVFPLAPSSKSTSGGTAALGCLVKDYFPEPVTVSWNSGALTSGVHTFPAVLQSSGLYSLSSVVTVPSSSLGTQTYICNVNHKPSNTKVDKRVEPKSCDKTHTCPPCPAPELLGGPSVFLFPPKPKDTLMISRTPEVTCVVVDVSHEDPEVKFNWYVDGVEVHNAKTKPREEQYNSTYRVVSVLTVLHQDWLNGKEYKCKVSNKALPAPIEKTISKAKGQPREPQVYTLPPSREEMTKNQVSLTCLVKGFYPSDIAVEWESNGQPENNYKTTPPVLDSDGSFFLYSKLTVDKSRWQQGNVFSCSVMHEALHNHYTQKSLSLSPGK

SEQ ID NO: 42 - DNA, 702 bp, Artificial Sequence
  Humanized Antibody
atggtgctgcagacccaggtgttcatctccctgctgctgtggatctccggcgcctacggcgacatccagatgacccagagcccttccagcctgtccgcttccgtgggcgacagagtgaccatcacctgtcaggcctccgaggacatctactccggcctggcctggtatcagcagaagcccggcaagtcccccaagctgctgatctacggcgctggatctctgcaggacggcgtgccctctagattctccggctctggatccggcacccactacaccctgaccatctccagcctgcagcccgaggacttcgctacctacttctgtcagcaaggcctgaagttccccctgaccttcggccagggcaccaaggtggaaatcaagcggaccgtggccgctccctccgtgtttatcttcccaccctccgacgagcagctgaagtccggcacagcttctgtcgtgtgcctgctgaacaacttctacccccgcgaggccaaggtgcagtggaaggtggacaacgccctgcagtccggcaactcccaggaatccgtgaccgagcaggactccaaggacagcacctactccctgtcctctaccctgaccctgtccaaggccgactacgagaagcacaaggtgtacgcctgcgaagtgacccaccagggcctgtctagccccgtgaccaagtctttcaaccggggcgagtgc

SEQ ID NO: 43 - protein, 234 aa, Artificial Sequence
  Humanized Antibody
MVLQTQVFISLLLWISGAYGDIQMTQSPSSLSASVGDRVTITCQASEDIYSGLAWYQQKPGKSPKLLIYGAGSLQDGVPSRFSGSGSGTHYTLTISSLQPEDFATYFCQQGLKFPLTFGQGTKVEIKRTVAAPSVFIFPPSDEQLKSGTASVVCLLNNFYPREAKVQWKVDNALQSGNSQESVTEQDSKDSTYSLSSTLTLSKADYEKHKVYACEVTHQGLSSPVTKSFNRGEC

SEQ ID NO: 44 - DNA, 34 bp, Artificial Sequence
  Primer F
cacggcaacctgctggagcggctgctgggggagg

SEQ ID NO: 45 - DNA, 24 bp, Artificial Sequence
  Primer R
caggctgttcccagacaggtccag